European Patent Specification EP 3 807 421 B1, published September 13, 2023. Title: Method for predicting a necrotic enteritis outbreak in an avian population. Applicant: Evonik Degussa GmbH. The sequence listing filed with the application follows.

SEQUENCE LISTING (8 sequences)

SEQ ID NO: 1 - DNA, 969 bp, Clostridium perfringens
  misc_feature (10)..(10): n is a, c, g, or t
  misc_feature (391)..(396): n is a, c, g, or t
  misc_feature (418)..(420): n is a, c, g, or t
  misc_feature (443)..(443): n is a, c, g, or t
  misc_feature (497)..(497): n is a, c, g, or t
  misc_feature (502)..(502): n is a, c, g, or t
ttgaaaagantaaaaattatttcaattacactagttcttacaagtgtaattagtacaagccttttttcaactcaaactcaagtttttgcaagtgaattaaatgacataaacaaaattgagttgaaaaatctaagtggagaaataataaaagaaaatggaaaggaagctattaaatatacttctagtgataccgcttcacataaaggttggaaggcaactttaagtggaacatttattgaagatcctcattctgataagaaaactgctttattaaatttagaaggatttataccttctgataaacagatttttggttctaaatattacggaaaaatgaaatggcctgaaacttatagaattaatgtaaaaagtgctgatgtaaataataatnnnnnnatagcaaattctattcctaaannnactatagataaaaaagatgtatntaattcaattggttattctataggcggtaatatatctgttgaaggaaaaactgntggtnctggaataaatgcttcatataatgtccaaaatactataagctatgaacaacctgattttagaacaattcaaagaaaagatgatgcaaatttagcatcatgggatataaaatttgttgagactaaggacggttataatatagattcttatcatgctatttatggaaatcaattattcatgaaatcaagattgtataataatggtgataaaaatttcacagatgatagagatttatcaacattaatttctggtggattttcacccaatatggctttagcattaacagcacctaaaaatgctaaagaatctgtaataatagttgaatatcaaagatttgataatgactatattttaaattgggaaactactcaatggcgaggaacaaacaaactttcgtcaacaagtgaatataacgaatttatgtttaaaataaattggcaagatcataaaatagaatattatctgtaa

SEQ ID NO: 2 - DNA, 1197 bp, Clostridium perfringens
  misc_feature (21)..(21): n is a, c, g, or t
  misc_feature (23)..(24): n is a, c, g, or t
  misc_feature (28)..(28): n is a, c, g, or t
  misc_feature (36)..(37): n is a, c, g, or t
  misc_feature (40)..(40): n is a, c, g, or t
  misc_feature (44)..(44): n is a, c, g, or t
  misc_feature (64)..(65): n is a, c, g, or t
  misc_feature (78)..(78): n is a, c, g, or t
  misc_feature (81)..(81): n is a, c, g, or t
  misc_feature (96)..(96): n is a, c, g, or t
  misc_feature (102)..(102): n is a, c, g, or t
  misc_feature (128)..(128): n is a, c, g, or t
  misc_feature (138)..(139): n is a, c, g, or t
  misc_feature (147)..(147): n is a, c, g, or t
  misc_feature (160)..(160): n is a, c, g, or t
  misc_feature (165)..(165): n is a, c, g, or t
  misc_feature (167)..(167): n is a, c, g, or t
  misc_feature (170)..(170): n is a, c, g, or t
  misc_feature (213)..(213): n is a, c, g, or t
  misc_feature (225)..(225): n is a, c, g, or t
  misc_feature (264)..(264): n is a, c, g, or t
  misc_feature (267)..(267): n is a, c, g, or t
  misc_feature (274)..(274): n is a, c, g, or t
  misc_feature (288)..(288): n is a, c, g, or t
  misc_feature (307)..(307): n is a, c, g, or t
  misc_feature (318)..(318): n is a, c, g, or t
  misc_feature (360)..(360): n is a, c, g, or t
  misc_feature (393)..(393): n is a, c, g, or t
  misc_feature (420)..(420): n is a, c, g, or t
  misc_feature (423)..(423): n is a, c, g, or t
  misc_feature (429)..(429): n is a, c, g, or t
  misc_feature (453)..(453): n is a, c, g, or t
  misc_feature (510)..(510): n is a, c, g, or t
  misc_feature (540)..(540): n is a, c, g, or t
  misc_feature (552)..(552): n is a, c, g, or t
  misc_feature (558)..(558): n is a, c, g, or t
  misc_feature (567)..(567): n is a, c, g, or t
  misc_feature (584)..(584): n is a, c, g, or t
  misc_feature (600)..(600): n is a, c, g, or t
  misc_feature (604)..(605): n is a, c, g, or t
  misc_feature (613)..(613): n is a, c, g, or t
  misc_feature (621)..(621): n is a, c, g, or t
  misc_feature (633)..(633): n is a, c, g, or t
  misc_feature (680)..(680): n is a, c, g, or t
  misc_feature (684)..(684): n is a, c, g, or t
  misc_feature (738)..(738): n is a, c, g, or t
  misc_feature (741)..(742): n is a, c, g, or t
  misc_feature (757)..(757): n is a, c, g, or t
  misc_feature (759)..(759): n is a, c, g, or t
  misc_feature (783)..(783): n is a, c, g, or t
  misc_feature (807)..(807): n is a, c, g, or t
  misc_feature (825)..(826): n is a, c, g, or t
  misc_feature (840)..(840): n is a, c, g, or t
  misc_feature (843)..(843): n is a, c, g, or t
  misc_feature (885)..(885): n is a, c, g, or t
  misc_feature (963)..(963): n is a, c, g, or t
  misc_feature (978)..(978): n is a, c, g, or t
  misc_feature (985)..(985): n is a, c, g, or t
  misc_feature (993)..(993): n is a, c, g, or t
  misc_feature (999)..(999): n is a, c, g, or t
  misc_feature (1014)..(1014): n is a, c, g, or t
  misc_feature (1020)..(1020): n is a, c, g, or t
  misc_feature (1087)..(1087): n is a, c, g, or t
  misc_feature (1094)..(1094): n is a, c, g, or t
  misc_feature (1117)..(1117): n is a, c, g, or t
  misc_feature (1124)..(1124): n is a, c, g, or t
  misc_feature (1143)..(1143): n is a, c, g, or t
  misc_feature (1149)..(1149): n is a, c, g, or t
  misc_feature (1158)..(1158): n is a, c, g, or t
atgaaaagaaagatttgtaangnncttntttgtgcnncgntagnaactagcctatgggctgggnnatcaactaaagtntangcttgggatggaaanattganggaacaggaactcatgctatgattgnaactcaaggnntttcaatnttagaaaatgatntgtcnanaantgaaccagaaagtgtaagaaaaaacttagagattttaaaaganaacatgcatgancttcaattaggttctacttatccagattatgataagaangcntatgatntatatcaagatcanttctgggatcctgatacanataataatttntcaaaggataatagttggtatttagcttattctatacctganacaggggaatcacaaataagaaaattttcagcnttagctagatatgaatggcaaagaggnaantataancaagctacattctatcttggagangctatgcactattttggagatatagatactccatatcatcctgctaatgttactgcngttgatagcgcaggacatgttaagtttganacttttgcagangaaagnaaagaacantataaaataaacacagnaggttgcaaaactaangagnntttttatnctgatatnttaaaaaacaangattttaatgcatggtcaaaagaatatgcaagaggttttgctaaaanaggnaaatcaatatactatagtcatgctagcatgagtcatagttgggatgattgggantanncagcaaaggtaactntngctaactctcaaaaaggaacagcnggatatatttatagattcttacangatgtatcagagggtaannatccatcagttggnaanaatgtaaaagaactagtagcttacatatcaactagtggtganaaagatgctggaacagatgactacatgtattttggaatcaaaacaaaggatggaaaaactcaagaatgggaaatgganaacccaggaaatgantttatgnctggaagnaaaganacttatactttcaanttaaangatgaaaatctaaaaattgatgatatacaaaatatgtggattagaaaaagaaaatatacagcattcncagatgnttataagccagaaaacataaagntaatagnaaatggaaaagttgtagtngacaangatataaangagtggatttcaggaaattcaacttataatataaaataa

SEQ ID NO: 3 - DNA, 20 bp, Artificial Sequence
  Primer
tatacttctagtgataccgc

SEQ ID NO: 4 - DNA, 20 bp, Artificial Sequence
  Primer
atcagaatgaggatcttcaa

SEQ ID NO: 5 - DNA, 23 bp, Artificial Sequence
  Probe
tcacataaaggttggaaggcaac

SEQ ID NO: 6 - DNA, 20 bp, Artificial Sequence
  Primer
tacatatcaactagtggtga

SEQ ID NO: 7 - DNA, 20 bp, Artificial Sequence
  Primer
attcttgagtttttccatcc

SEQ ID NO: 8 - DNA, 27 bp, Artificial Sequence
  Probe
tggaacagatgactacatgtattttgg